European Patent Application EP 4 556 017 A1, published May 21, 2025. Title: 乙型肝炎病毒受体OATP及其应用. Applicant: 上海贺普药业股份有限公司. The sequence listing filed with the application follows.

SEQUENCE LISTING (182 sequences)

SEQ ID NO: 1 - protein, 702 aa, Homo sapiens
MDQHQHLNKTAESASSEKKKTRRCNGFKMFLAALSFSYIAKALGGIIMKISITQIERRFDISSSLAGLIDGSFEIGNLLVIVFVSYFGSKLHRPKLIGIGCLLMGTGSILTSLPHFFMGYYRYSKETHINPSENSTSSLSTCLINQTLSFNGTSPEIVEKDCVKESGSHMWIYVFMGNMLRGIGETPIVPLGISYIDDFAKEGHSSLYLGSLNAIGMIGPVIGFALGSLFAKMYVDIGYVDLSTIRITPKDSRWVGAWWLGFLVSGLFSIISSIPFFFLPKNPNKPQKERKISLSLHVLKTNDDRNQTANLTNQGKNVTKNVTGFFQSLKSILTNPLYVIFLLLTLLQVSSFIGSFTYVFKYMEQQYGQSASHANFLLGIITIPTVATGMFLGGFIIKKFKLSLVGIAKFSFLTSMISFLFQLLYFPLICESKSVAGLTLTYDGNNSVASHVDVPLSYCNSECNCDESQWEPVCGNNGITYLSPCLAGCKSSSGIKKHTVFYNCSCVEVTGLQNRNYSAHLGECPRDNTCTRKFFIYVAIQVINSLFSATGGTTFILLTVKIVQPELKALAMGFQSMVIRTLGGILAPIYFGALIDKTCMKWSTNSCGAQGACRIYNSVFFGRVYLGLSIALRFPALVLYIVFIFAMKKKFQGKDTKASDNERKVMDEANLEFLNNGEHFVPSAGTDSKTCNLDMQDNAAAN

SEQ ID NO: 2 - DNA, 2109 bp, Homo sapiens
  source 1..2109: mol_type = genomic DNA
atggaccaacatcaacatttgaataaaacagcagagtcagcatcttcagagaaaaagaaaacaagacgctgcaatggattcaagatgttcttggcagccctgtcattcagctatattgctaaagcactaggtggaatcattatgaaaatttccatcactcaaatagaaaggagatttgacatatcctcttctcttgctggtttaattgatggaagctttgaaattggaaatttgcttgtgattgtatttgtaagttactttggatctaaactacacagaccgaagttaattggaattggttgtctccttatgggaactggaagtattttgacatctttaccacatttcttcatgggatattataggtattctaaagaaacccatattaatccatcagaaaattcaacatcaagtttatcaacctgtttaattaatcaaaccttatcattcaatggaacatcacctgagatagtagaaaaagattgtgtaaaggaatctgggtcacacatgtggatctatgtcttcatggggaatatgcttcgtggcataggggaaacccccatagtaccattggggatttcatacattgatgattttgcaaaagaaggacattcttccttgtatttaggtagtttgaatgcaataggaatgattggtccagtcattggctttgcactgggatctctgtttgctaaaatgtacgtggatattggatatgtagatctgagcactatcagaataactcctaaggactctcgttgggttggagcttggtggcttggtttccttgtgtctggactattttccattatttcttccataccattttttttcttgccgaaaaatccaaataaaccacaaaaagaaagaaaaatttcactatcattgcatgtgctgaaaacaaatgatgatagaaatcaaacagctaatttgaccaaccaaggaaaaaatgttaccaaaaatgtgactggttttttccagtctttgaaaagcatccttaccaatcccctgtatgttatatttctgcttttgacattgttacaagtaagcagctttattggttcttttacttacgtctttaaatatatggagcaacagtacggtcagtctgcatctcatgctaactttttgttgggaatcataaccattcctacggttgcaactggaatgtttttaggaggatttatcattaaaaaattcaaattgtctttagttggaattgccaaattttcatttcttacttcgatgatatccttcttgtttcaacttctatatttccctctaatctgcgaaagcaaatcagttgccggcctaaccttgacctatgatggaaataattcagtggcatctcatgtagatgtaccactttcttattgcaactcagagtgcaattgtgatgaaagtcagtgggaaccagtctgtgggaacaatggaataacttacctgtcaccttgtctagcaggatgcaaatcctcaagtggtattaaaaagcatacagtgttttataactgtagttgtgtggaagtaactggtctccagaacagaaattactcagcacacttgggtgaatgcccaagagataatacttgtacaaggaaatttttcatctatgttgcaattcaagtcataaactctttgttctctgcaacaggaggtaccacatttatcttgttgactgtgaagattgttcaacctgaattgaaagcacttgcaatgggtttccagtcaatggttataagaacactaggaggaattctagctccaatatattttggggctctgattgataaaacatgtatgaagtggtccaccaacagctgtggagcacaaggggcttgtaggatatataattccgtattttttggaagggtctacttgggcttatctatagctttaagattcccagcacttgttttatatattgttttcatttttgctatgaagaaaaaatttcaaggaaaagataccaaggcatcggacaatgaaagaaaagtaatggatgaagcaaacttagaattcttaaataatggtgaacattttgtaccttctgctggaacagatagtaaaacatgtaatttggacatgcaagacaatgctgctgccaactaa

SEQ ID NO: 3 - DNA, 3013 bp, Homo sapiens
  source 1..3013: mol_type = genomic DNA
agactttaacatcagaaaaaggatggacttgttgcagttgctgtagcattcaaagtcaagttgtgctttgcgatgctgagtttactgttttaaatggacttcaagcatagccctgaagtgttgtcccgttgttcccacctcctagagggcctgacagaagaggtacatatgctatgtgatcatttcaaaccaagcatcagcaacaattaaaaatattcacttggtatctgtagtttaataatggaccaacatcaacatttgaataaaacagcagagtcagcatcttcagagaaaaagaaaacaagacgctgcaatggattcaagatgttcttggcagccctgtcattcagctatattgctaaagcactaggtggaatcattatgaaaatttccatcactcaaatagaaaggagatttgacatatcctcttctcttgctggtttaattgatggaagctttgaaattggaaatttgcttgtgattgtatttgtaagttactttggatctaaactacacagaccgaagttaattggaattggttgtctccttatgggaactggaagtattttgacatctttaccacatttcttcatgggatattataggtattctaaagaaacccatattaatccatcagaaaattcaacatcaagtttatcaacctgtttaattaatcaaaccttatcattcaatggaacatcacctgagatagtagaaaaagattgtgtaaaggaatctgggtcacacatgtggatctatgtcttcatggggaatatgcttcgtggcataggggaaacccccatagtaccattggggatttcatacattgatgattttgcaaaagaaggacattcttccttgtatttaggtagtttgaatgcaataggaatgattggtccagtcattggctttgcactgggatctctgtttgctaaaatgtacgtggatattggatatgtagatctgagcactatcagaataactcctaaggactctcgttgggttggagcttggtggcttggtttccttgtgtctggactattttccattatttcttccataccattttttttcttgccgaaaaatccaaataaaccacaaaaagaaagaaaaatttcactatcattgcatgtgctgaaaacaaatgatgatagaaatcaaacagctaatttgaccaaccaaggaaaaaatgttaccaaaaatgtgactggttttttccagtctttgaaaagcatccttaccaatcccctgtatgttatatttctgcttttgacattgttacaagtaagcagctttattggttcttttacttacgtctttaaatatatggagcaacagtacggtcagtctgcatctcatgctaactttttgttgggaatcataaccattcctacggttgcaactggaatgtttttaggaggatttatcattaaaaaattcaaattgtctttagttggaattgccaaattttcatttcttacttcgatgatatccttcttgtttcaacttctatatttccctctaatctgcgaaagcaaatcagttgccggcctaaccttgacctatgatggaaataattcagtggcatctcatgtagatgtaccactttcttattgcaactcagagtgcaattgtgatgaaagtcagtgggaaccagtctgtgggaacaatggaataacttacctgtcaccttgtctagcaggatgcaaatcctcaagtggtattaaaaagcatacagtgttttataactgtagttgtgtggaagtaactggtctccagaacagaaattactcagcacacttgggtgaatgcccaagagataatacttgtacaaggaaatttttcatctatgttgcaattcaagtcataaactctttgttctctgcaacaggaggtaccacatttatcttgttgactgtgaagattgttcaacctgaattgaaagcacttgcaatgggtttccagtcaatggttataagaacactaggaggaattctagctccaatatattttggggctctgattgataaaacatgtatgaagtggtccaccaacagctgtggagcacaaggggcttgtaggatatataattccgtattttttggaagggtctacttgggcttatctatagctttaagattcccagcacttgttttatatattgttttcatttttgctatgaagaaaaaatttcaaggaaaagataccaaggcatcggacaatgaaagaaaagtaatggatgaagcaaacttagaattcttaaataatggtgaacattttgtaccttctgctggaacagatagtaaaacatgtaatttggacatgcaagacaatgctgctgccaactaacattgcattgattcattaagatgttatttttgaggtgttcctggtctttcactgacaattccaacattctttacttacagtggaccaatggataagtctatgcatctataataaactataaaaaatgggagtacccatggttaggatatagctatgcctttatggttaagattagaatatatgatccataaaaatttaaagtgagaggcatggttagtgtgtgatacaataaaaagtaattgtttggtagttgtaactgctaataaaaccagtgactagaatataagggaggtaaaaaggacaagatagattaatagcctaaataaagagaaaagcctgatgcctttaaaaaaaatgaaacactttggatgtattacttaggccaaaatctggcctggatttatgctataatatatattttcatgttaagttgtatatttttcagaaattataaatattattaatttaaaatttgaatttgtgtttgactaacaacctcgatggatcttcttccaacctcccattaagatcctgcagaagaaatagaaatattcaaatattgcaaggtgtaattgtgagacaacttattataatacgtgttaagtttctactggacccatggaagtggattaagaaaaaccgactttagcttgagaaagcaaaa

SEQ ID NO: 4 - protein, 691 aa, Homo sapiens
MDQNQHLNKTAEAQPSENKKTRYCNGLKMFLAALSLSFIAKTLGAIIMKSSIIHIERRFEISSSLVGFIDGSFEIGNLLVIVFVSYFGSKLHRPKLIGIGCFIMGIGGVLTALPHFFMGYYRYSKETNINSSENSTSTLSTCLINQILSLNRASPEIVGKGCLKESGSYMWIYVFMGNMLRGIGETPIVPLGLSYIDDFAKEGHSSLYLGILNAIAMIGPIIGFTLGSLFSKMYVDIGYVDLSTIRITPTDSRWVGAWWLNFLVSGLFSIISSIPFFFLPQTPNKPQKERKASLSLHVLETNDEKDQTANLTNQGKNITKNVTGFFQSFKSILTNPLYVMFVLLTLLQVSSYIGAFTYVFKYVEQQYGQPSSKANILLGVITIPIFASGMFLGGYIIKKFKLNTVGIAKFSCFTAVMSLSFYLLYFFILCENKSVAGLTMTYDGNNPVTSHRDVPLSYCNSDCNCDESQWEPVCGNNGITYISPCLAGCKSSSGNKKPIVFYNCSCLEVTGLQNRNYSAHLGECPRDDACTRKFYFFVAIQVLNLFFSALGGTSHVMLIVKIVQPELKSLALGFHSMVIRALGGILAPIYFGALIDTTCIKWSTNNCGTRGSCRTYNSTSFSRVYLGLSSMLRVSSLVLYIILIYAMKKKYQEKDINASENGSVMDEANLESLNKNKHFVPSAGADSETHC

SEQ ID NO: 5 - DNA, 2076 bp, Homo sapiens
  source 1..2076: mol_type = genomic DNA
atggaccaaaatcaacatttgaataaaacagcagaggcacaaccttcagagaataagaaaacaagatactgcaatggattgaagatgttcttggcagctctgtcactcagctttattgctaagacactaggtgcaattattatgaaaagttccatcattcatatagaacggagatttgagatatcctcttctcttgttggttttattgacggaagctttgaaattggaaatttgcttgtgattgtatttgtgagttactttggatccaaactacatagaccaaagttaattggaatcggttgtttcattatgggaattggaggtgttttgactgctttgccacatttcttcatgggatattacaggtattctaaagaaactaatatcaattcatcagaaaattcaacatcgaccttatccacttgtttaattaatcaaattttatcactcaatagagcatcacctgagatagtgggaaaaggttgtttaaaggaatctgggtcatacatgtggatatatgtgttcatgggtaatatgcttcgtggaataggggagactcccatagtaccattggggctttcttacattgatgatttcgctaaagaaggacattcttctttgtatttaggtatattgaatgcaatagcaatgattggtccaatcattggctttaccctgggatctctgttttctaaaatgtacgtggatattggatatgtagatctaagcactatcaggataactcctactgattctcgatgggttggagcttggtggcttaatttccttgtgtctggactattctccattatttcttccataccattctttttcttgccccaaactccaaataaaccacaaaaagaaagaaaagcttcactgtctttgcatgtgctggaaacaaatgatgaaaaggatcaaacagctaatttgaccaatcaaggaaaaaatattaccaaaaatgtgactggttttttccagtcttttaaaagcatccttactaatcccctgtatgttatgtttgtgcttttgacgttgttacaagtaagcagctatattggtgcttttacttatgtcttcaaatacgtagagcaacagtatggtcagccttcatctaaggctaacatcttattgggagtcataaccatacctatttttgcaagtggaatgtttttaggaggatatatcattaaaaaattcaaactgaacaccgttggaattgccaaattctcatgttttactgctgtgatgtcattgtccttttacctattatattttttcatactctgtgaaaacaaatcagttgccggactaaccatgacctatgatggaaataatccagtgacatctcatagagatgtaccactttcttattgcaactcagactgcaattgtgatgaaagtcaatgggaaccagtctgtggaaacaatggaataacttacatctcaccctgtctagcaggttgcaaatcttcaagtggcaataaaaagcctatagtgttttacaactgcagttgtttggaagtaactggtctccagaacagaaattactcagcccatttgggtgaatgcccaagagatgatgcttgtacaaggaaattttacttttttgttgcaatacaagtcttgaatttatttttctctgcacttggaggcacctcacatgtcatgctgattgttaaaattgttcaacctgaattgaaatcacttgcactgggtttccactcaatggttatacgagcactaggaggaattctagctccaatatattttggggctctgattgatacaacgtgtataaagtggtccaccaacaactgtggcacacgtgggtcatgtaggacatataattccacatcattttcaagggtctacttgggcttgtcttcaatgttaagagtctcatcacttgttttatatattatattaatttatgccatgaagaaaaaatatcaagagaaagatatcaatgcatcagaaaatggaagtgtcatggatgaagcaaacttagaatccttaaataaaaataaacattttgtcccttctgctggggcagatagtgaaacacattgttaa

SEQ ID NO: 6 - DNA, 2787 bp, Homo sapiens
  source 1..2787: mol_type = genomic DNA
aaagggtggacttgttgcagttgctgtaggattctaaatccaggtgattgtttcaaactgagcatcaacaacaaaaacatttgtatgatatctatatttcaatcatggaccaaaatcaacatttgaataaaacagcagaggcacaaccttcagagaataagaaaacaagatactgcaatggattgaagatgttcttggcagctctgtcactcagctttattgctaagacactaggtgcaattattatgaaaagttccatcattcatatagaacggagatttgagatatcctcttctcttgttggttttattgacggaagctttgaaattggaaatttgcttgtgattgtatttgtgagttactttggatccaaactacatagaccaaagttaattggaatcggttgtttcattatgggaattggaggtgttttgactgctttgccacatttcttcatgggatattacaggtattctaaagaaactaatatcaattcatcagaaaattcaacatcgaccttatccacttgtttaattaatcaaattttatcactcaatagagcatcacctgagatagtgggaaaaggttgtttaaaggaatctgggtcatacatgtggatatatgtgttcatgggtaatatgcttcgtggaataggggagactcccatagtaccattggggctttcttacattgatgatttcgctaaagaaggacattcttctttgtatttaggtatattgaatgcaatagcaatgattggtccaatcattggctttaccctgggatctctgttttctaaaatgtacgtggatattggatatgtagatctaagcactatcaggataactcctactgattctcgatgggttggagcttggtggcttaatttccttgtgtctggactattctccattatttcttccataccattctttttcttgccccaaactccaaataaaccacaaaaagaaagaaaagcttcactgtctttgcatgtgctggaaacaaatgatgaaaaggatcaaacagctaatttgaccaatcaaggaaaaaatattaccaaaaatgtgactggttttttccagtcttttaaaagcatccttactaatcccctgtatgttatgtttgtgcttttgacgttgttacaagtaagcagctatattggtgcttttacttatgtcttcaaatacgtagagcaacagtatggtcagccttcatctaaggctaacatcttattgggagtcataaccatacctatttttgcaagtggaatgtttttaggaggatatatcattaaaaaattcaaactgaacaccgttggaattgccaaattctcatgttttactgctgtgatgtcattgtccttttacctattatattttttcatactctgtgaaaacaaatcagttgccggactaaccatgacctatgatggaaataatccagtgacatctcatagagatgtaccactttcttattgcaactcagactgcaattgtgatgaaagtcaatgggaaccagtctgtggaaacaatggaataacttacatctcaccctgtctagcaggttgcaaatcttcaagtggcaataaaaagcctatagtgttttacaactgcagttgtttggaagtaactggtctccagaacagaaattactcagcccatttgggtgaatgcccaagagatgatgcttgtacaaggaaattttacttttttgttgcaatacaagtcttgaatttatttttctctgcacttggaggcacctcacatgtcatgctgattgttaaaattgttcaacctgaattgaaatcacttgcactgggtttccactcaatggttatacgagcactaggaggaattctagctccaatatattttggggctctgattgatacaacgtgtataaagtggtccaccaacaactgtggcacacgtgggtcatgtaggacatataattccacatcattttcaagggtctacttgggcttgtcttcaatgttaagagtctcatcacttgttttatatattatattaatttatgccatgaagaaaaaatatcaagagaaagatatcaatgcatcagaaaatggaagtgtcatggatgaagcaaacttagaatccttaaataaaaataaacattttgtcccttctgctggggcagatagtgaaacacattgttaaggggagaaaaaaagccacttctgcttctgtgtttccaaacagcattgcattgattcagtaagatgttatttttgaggagttcctggtcctttcactaagaatttccacatcttttatggtggaagtataaataagcctatgaacttataataaaacaaactgtaggtagaaaaaatgagagtactcattgttacattatagctacatatttgtggttaaggttagactatatgatccatacaaattaaagtgagagacatggttactgtgtaataaaagaaaaaatacttgttcaggtaattctaattcttaataaaacaaatgagtatcatacaggtagaggttaaaaaggaggagctagattcatatcctaagtaaagagaaatgcctagtgtctattttattaaacaaacaaacacagagtttgaactataatactaaggcctgaagtctagcttggatatatgctacaataatatctgttactcacataaaattatatatttcacagactttatcaatgtataattaacaattatcttgtttaagtaaatttagaatacatttaagtattgtggaagaaataaagacattccaatatttgcaa

SEQ ID NO: 7 - protein, 349 aa, Homo sapiens
MEAHNASAPFNFTLPPNFGKRPTDLALSVILVFMLFFIMLSLGCTMEFSKIKAHLWKPKGLAIALVAQYGIMPLTAFVLGKVFRLKNIEALAILVCGCSPGGNLSNVFSLAMKGDMNLSIVMTTCSTFCALGMMPLLLYIYSRGIYDGDLKDKVPYKGIVISLVLVLIPCTIGIVLKSKRPQYMRYVIKGGMIIILLCSVAVTVLSAINVGKSIMFAMTPLLIATSSLMPFIGFLLGYVLSALFCLNGRCRRTVSMETGCQNVQLCSTILNVAFPPEVIGPLFFFPLLYMIFQLGEGLLLIAIFWCYEKFKTPKDKTKMIYTAATTEETIPGALGNGTYKGEDCSPCTA

SEQ ID NO: 8 - protein, 163 aa, Duck hepatitis B virus
MGQQPAKSMDVRRIEGGELLLNQLAGRMIPKGTVTWSGKFPTIDHLLDHVQTMEEVNTLQQQGAWPAGAGRRLGLTNPTPHETPQPQWTPEEDQKAREAFRRYQEERPPETTTIAPTSPTPWKLQPGDDPLLENKSLLETHPLYQNPEPAVPVIKTPPLKKKK

SEQ ID NO: 9 - protein, 166 aa, Heron hepatitis B virus
MGHTQAKSTTDRRVEGGELLLQHLAGRMIPPEFSGPITTAGKFPTIQHVMDHIDSVEELRTLQAGGHWPEGTARRLGLDQPRPTPPPITWTEEEDKKAKEFFKQYQENRPKPAETAPPPITELHAAEPPQWKISPEDPLLKAKALIPVKEPEVPILKVPKLTNKKK

SEQ ID NO: 10 - protein, 108 aa, Woolly monkey hepatitis B virus
MGLNQSTFNPLGFFPSHQLDPLFKANAGSADWDKNPNKDPWPQAHDTAVGAFGPGLVPPHGGLLGWSSQAQGLSVTVPDTPPPPSTNRDKGRKPTPATPPLRDTHPQA

SEQ ID NO: 11 - protein, 108 aa, Capuchin monkey hepatitis B virus
MGLNQSTINPLGFFPSHQLDPLFKANSPAADWDQNPHKDPWPSAHEVPVGAFGPGLVPPHGGLLGWNPQSQGQVTLLPKDPPAQLPNRNSARVPTPITPPLRDTHPQA

SEQ ID NO: 12 - protein, 149 aa, Woodchuck hepatitis virus
MGNNIKVTFNPDKIAAWWPAVGTYYTTTYPQNQSVFQPGIYQTTSLINPKNQQELDSVLINRYKQIDWNTWQGFPVDQKLPLVSRDPPPKPYINQSAQTFEIKPGPIIVPGIRDIPRGLVPPQTPTNRDQGRKPTPPTPPLRDTHPHLT

SEQ ID NO: 13 - protein, 132 aa, Ground squirrel hepatitis virus
MKNQTGHLQGFAEGLRALTTSDHHNSAYGDPFTTLSPVVPTVSTTLSPPLTIGDPVLSTEMSPSGLLGLLAGLQVVYFLWTKILTIAQSLDWWWTSLSFPGGIPECTGQNLQFQTCKHLPTSCPPTCNGFRW

SEQ ID NO: 14 - protein, 130 aa, Hepatitis B virus
MGQNWSIPNPLGFLPEHQLPNPYAPVYQDWDLNQDKDQWPQAREVSPGAYGLGFVPPHGGLTGNLPFAQEGNLTSNNPETIVYQIPKAKDESQTQVIQLPAPPRTTTNRKKGRQPTPPTPPVRVTHPHLN

SEQ ID NO: 15 - protein, 119 aa, Hepatitis B virus
MGGWSSKPRKGMGTNLSVPNPLGFFPDHQLDPAFGANSNNPDWDFNPIKDHWPAGNQVGVGAFGPRLTPPHGGILGWSPQAQGILATVSTIPPPASTNRQSGRQPTPISPPLRDSHPEA

SEQ ID NO: 16 - protein, 119 aa, Hepatitis B virus
MGGWSSKPRKGMGTNLSVPNPLGFFPDHQLDPAFKANSENPDWDLNPHKDNWPDANKVGVGAFGPGFTPPHGGLLGWSPQAQGLLTTVPAAPPPASTNRQSGRQPTPLSPPLRDTHPQA

SEQ ID NO: 17 - protein, 119 aa, Hepatitis B virus
MGGWSSKPRQGMGTNLSVPNPLGFFPDHQLDPAFGANSNNPDWDFNPNKDHWPEANQVGAGAFGPGFTPPHGGLLGWSPQAQGILTTVPVAPPPASTNRQSGRQPTPISPPLRDSHPQA

SEQ ID NO: 18 - protein, 108 aa, Hepatitis B virus
MGQNLSTSNPLGFFPDHQLDPAFRANTANPDWDFNPNKDTWPDANKVGAGAFGLGFTPPHGGLLGWSPQAQGILQTLPANPPPASTHRQSGRQPTPLSPPLRNTHPQA

SEQ ID NO: 19 - protein, 118 aa, Hepatitis B virus
MGLSWTVPLEWGKNHSTTNPLGFFPDHQLDPAFRANTRNPDWDHNPDKDHWTEANKVGVGAFGPGFTPPHGGLLGWSPQAQGMLKTLPADPPPASTNRQSGRQPTPITPPLRDTHPQA

SEQ ID NO: 20 - protein, 119 aa, Hepatitis B virus
MGAPLSTTRRGMGQNLSVPNPLGFFPDHQLDPLFRANSSSPDWDFNKNKDNWPMANKVGVGGYGPGFTPPHGGLLGWSPQAQGVLTTLPADPPPASTNRRSGRKPTPVSPPLRDTHPQA

SEQ ID NO: 21 - protein, 118 aa, Hepatitis B virus
MGLSWTVPLEWGKNLSTSNPLGFLPDHQLDPAFRANTNNPDWDFNPKKDPWPEANKVGVGAYGPGFTPPHGGLLGWSLQSQGTLTTLPADPPPASTNRQSGRQPTPISPPLRDSHPQA

SEQ ID NO: 22 - protein, 119 aa, Hepatitis B virus
MGAPLSTARRGMGQNLSVPNPLGFFPDHQLDPLFRANSSSPDWDFNTNKDNWPMANKVGVGGFGPGFTPPHGGLLGWSPQAQGILTTSPPDPPPASTNRRSGRKPTPVSPPLRDTHPQA

SEQ ID NO: 23 - protein, 118 aa, synthetic construct
GGWSSKPRQGMGTNLSVPNPLGFFPDHQLDPAFGANSNNPDWDFNPNKDHWPEANQVGAGAFGPGFTPPHGGLLGWSPQAQGILTTVPVAPPPASTNRQSGRQPTPISPPLRDSHPQA

SEQ ID NO: 24 - protein, 68 aa, synthetic construct
GGWSSKPRQGMGTNLSVPNPLGFFPDHQLDPAFGANSNNPDWDFNPNKDHWPEANQVGAGAFGPGFTP

SEQ ID NO: 25 - protein, 58 aa, synthetic construct
GGWSSKPRQGMGTNLSVPNPLGFFPDHQLDPAFGANSNNPDWDFNPNKDHWPEANQVG

SEQ ID NO: 26 - protein, 107 aa, synthetic construct
GTNLSVPNPLGFFPDHQLDPAFGANSNNPDWDFNPNKDHWPEANQVGAGAFGPGFTPPHGGLLGWSPQAQGILTTVPVAPPPASTNRQSGRQPTPISPPLRDSHPQA

SEQ ID NO: 27 - protein, 76 aa, synthetic construct
GTNLSVPNPLGFFPDHQLDPAFGANSNNPDWDFNPNKDHWPEANQVGAGAFGPGFTPPHGGLLGWSPQAQGILTTV

SEQ ID NO: 28 - protein, 60 aa, synthetic construct
GTNLSVPNPLGFFPDHQLDPAFGANSNNPDWDFNPNKDHWPEANQVGAGAFGPGFTPPHG

SEQ ID NO: 29 - protein, 55 aa, synthetic construct
GTNLSVPNPLGFFPDHQLDPAFGANSNNPDWDFNPNKDHWPEANQVGAGAFGPGF

SEQ ID NO: 30 - protein, 47 aa, synthetic construct
GTNLSVPNPLGFFPDHQLDPAFGANSNNPDWDFNPNKDHWPEANQVG

SEQ ID NO: 31 - protein, 40 aa, synthetic construct
GTNLSVPNPLGFFPDHQLDPAFGANSNNPDWDFNPNKDHW

SEQ ID NO: 32 - protein, 35 aa, synthetic construct
GTNLSVPNPLGFFPDHQLDPAFGANSNNPDWDFNP

SEQ ID NO: 33 - protein, 30 aa, synthetic construct
GTNLSVPNPLGFFPDHQLDPAFGANSNNPD

SEQ ID NO: 34 - protein, 25 aa, synthetic construct
GTNLSVPNPLGFFPDHQLDPAFGAN

SEQ ID NO: 35 - protein, 20 aa, synthetic construct
GTNLSVPNPLGFFPDHQLDP

SEQ ID NO: 36 - protein, 47 aa, synthetic construct
GTNLSVPNPLGFFPDHQLDPAFGANSNNPDWDFNPVKDDWPAANQVG

SEQ ID NO: 37 - protein, 47 aa, synthetic construct
GTNLSVPNPLGFFPDHQLDPAFKANSENPDWDLNPNKDNWPDANKVG

SEQ ID NO: 38 - protein, 47 aa, synthetic construct
GQNLSTSNPLGFFPDHQLDPAFRANTANPDWDFNPNKDTWPDANKVG

SEQ ID NO: 39 - protein, 47 aa, synthetic construct
GKNISTTNPLGFFPDHQLDPAFRANTRNPDWDHNPNKDHWTEANKVG

SEQ ID NO: 40 - protein, 47 aa, synthetic construct
GQNLSVPNPLGFFPDHQLDPLFRANSSSPDWDFNTNKDSWPMANKVG

SEQ ID NO: 41 - protein, 47 aa, synthetic construct
GKNLSASNPLGFLPDHQLDPAFRANTNNPDWDFNPKKDPWPEANKVG

SEQ ID NO: 42 - protein, 47 aa, synthetic construct
GQNLSVPNPLGFFPDHQLDPLFRANSSSPDWDFNTNKDNWPMANKVG

SEQ ID NO: 43 - protein, 47 aa, synthetic construct
GTDLSVPNPLGFFPDHQLDPAFGANSNNPDWDFNPNKDHWPEANQVG

SEQ ID NO: 44 - protein, 46 aa, synthetic construct
GTNLSVPNPLGFLPDHQLDPAFGANSNNPDDFNPNKDHWPEANQVG

SEQ ID NO: 45 - protein, 47 aa, synthetic construct
GTNLSVPNPLGFFPDHQLDPAFKANSNNPDWDFNPNKDHWPEANQVG

SEQ ID NO: 46 - protein, 47 aa, synthetic construct
GTNLSVPNPLGFFPDHQLDPAFGANSENPDWDFNPNKDHWPEANQVG

SEQ ID NO: 47 - protein, 47 aa, synthetic construct
GTNLSVPNPLGFFPDHQLDPAFGANSNNPDWDFKPNKDHWPEANQVG

SEQ ID NO: 48 - protein, 47 aa, synthetic construct
GTNLSVPNPLGFFPDHQLDPAFGANSNNPDWDLNPNKDHWPEANQVG

SEQ ID NO: 49 - protein, 47 aa, synthetic construct
GTNLSVPNPLGFFPDHQLDPAFGANSNNPDWDFNPHKDHWPEANQVG

SEQ ID NO: 50 - protein, 47 aa, synthetic construct
GTNLSVPNPLGFFPDHQLDPAFGANSNNPDWDFNPYKDHWPEANQVG

SEQ ID NO: 51 - protein, 47 aa, synthetic construct
GTNLSVPNPLGFFPDHQLDPAFGANSNNPDWDFNPKKDHWPEANQVG

SEQ ID NO: 52 - protein, 47 aa, synthetic construct
GTNLSVPNPLGFFPDHQLDPAFGANSNNPDWDFNPNKAHWPEANQVG

SEQ ID NO: 53 - protein, 47 aa, synthetic construct
GTNLSVPNPLGFFPDHQLDPAFGANSNNPDWDFNPNKDQWPEANQVG

SEQ ID NO: 54 - protein, 47 aa, synthetic construct
GTNLSVPNPLGFFPDHQLDPAFGANSNNPDWDFNPNKDNWPEANQVG

SEQ ID NO: 55 - protein, 47 aa, synthetic construct
GTNLSVPNPLGFFPDHQLDPAFGANSNNPDWDFNPNKDHWPKANQVG

SEQ ID NO: 56 - protein, 47 aa, synthetic construct
GTNLSVPNPLGFFPDHQLDPAFGANSNNPDWDFNPNKDHWPDANQVG

SEQ ID NO: 57 - protein, 47 aa, synthetic construct
GTNLSVPNPLGFFPDHQLDPAFGANSNNPDWDFNPNKDHWPESNQVG

SEQ ID NO: 58 - protein, 47 aa, synthetic construct
GTNLSVPNPLGFFPDHQLDPAFGANSNNPDWDFNPNKDHWPEAKQVG

SEQ ID NO: 59 - protein, 47 aa, synthetic construct
GTNLSVPNPLGFFPDHQLDPAFGANSNNPDWDFNPNKDHWPEADQVG

SEQ ID NO: 60 - protein, 47 aa, synthetic construct
GTNLSVPNPLGFFPDHQLDPAFGANSNNPDWDFNPNKDHWPEANKVG

SEQ ID NO: 61 - protein, 58 aa, synthetic construct
GGWSSKPRKGMGTNLSVPNPLGFFPDHQLDPAFGANSNNPDWDFNPNKDHWPEANQVG

SEQ ID NO: 62 - protein, 58 aa, synthetic construct; identical to SEQ ID NO: 61

SEQ ID NO: 63 - protein, 57 aa, synthetic construct
GLSWTVPLEWGTNLSVPNPLGFFPDHQLDPAFGANSNNPDWDFNPNKDHWPEANQVG

SEQ ID NO: 64 - protein, 58 aa, synthetic construct
GAPLSTTRRGMGTNLSVPNPLGFFPDHQLDPAFGANSNNPDWDFNPNKDHWPEANQVG

SEQ ID NO: 65 - protein, 57 aa, synthetic construct; identical to SEQ ID NO: 63

SEQ ID NO: 66 - protein, 58 aa, synthetic construct
GAPLSTARRGMGTNLSVPNPLGFFPDHQLDPAFGANSNNPDWDFNPNKDHWPEANQVG

SEQ ID NO: 67 - protein, 47 aa, synthetic construct; identical to SEQ ID NO: 30
  source 1..47: note = N-terminal modification with myristic acid and C-terminal modification with amination

SEQ ID NO: 68 - protein, 47 aa, synthetic construct; identical to SEQ ID NO: 60
  source 1..47: note = N-terminal modification with myristic acid and C-terminal modification with amination

SEQ ID NO: 69 - protein, 47 aa, synthetic construct; identical to SEQ ID NO: 30
  source 1..47: note = N-terminal modification with palmitic acid and C-terminal modification with amination

SEQ ID NO: 70 - protein, 47 aa, synthetic construct; identical to SEQ ID NO: 30
  source 1..47: note = N-terminal modification with stearic acid and C-terminal modification with amination

SEQ ID NO: 71 - protein, 47 aa, synthetic construct; identical to SEQ ID NO: 30
  source 1..47: note = N-terminal modification with cholesterol and C-terminal modification with amination

SEQ ID NO: 72 - protein, 47 aa, synthetic construct; identical to SEQ ID NO: 36
  source 1..47: note = N-terminal modification with myristic acid and C-terminal modification with amination

SEQ ID NO: 73 - protein, 47 aa, synthetic construct; identical to SEQ ID NO: 37
  source 1..47: note = N-terminal modification with myristic acid and C-terminal modification with amination

SEQ ID NO: 74 - protein, 47 aa, synthetic construct; identical to SEQ ID NO: 38
  source 1..47: note = N-terminal modification with myristic acid and C-terminal modification with amination

SEQ ID NO: 75 - protein, 47 aa, synthetic construct; identical to SEQ ID NO: 39
  source 1..47: note = N-terminal modification with myristic acid and C-terminal modification with amination

SEQ ID NO: 76 - protein, 47 aa, synthetic construct; identical to SEQ ID NO: 40
  source 1..47: note = N-terminal modification with myristic acid and C-terminal modification with amination

SEQ ID NO: 77 - protein, 47 aa, synthetic construct; identical to SEQ ID NO: 41
  source 1..47: note = N-terminal modification with myristic acid and C-terminal modification with amination

SEQ ID NO: 78 - protein, 47 aa, synthetic construct; identical to SEQ ID NO: 42
  source 1..47: note = N-terminal modification with myristic acid and C-terminal modification with amination

SEQ ID NO: 79 - DNA, 2002 bp, Homo sapiens
  source 1..2002: mol_type = genomic DNA
gattaaagaaggcatccagcaagaactgcacaagaaacggagtcagccggagaacaaggagtggtcttccactgcctcacaggaggatggaggcccacaacgcgtctgccccattcaacttcaccctgccacccaactttggcaagcgccccacagacctggcactgagcgtcatcctggtgttcatgttgttcttcatcatgctctcgctgggctgcaccatggagttcagcaagatcaaggctcacttatggaagcctaaagggctggccatcgccctggtggcacagtatggcatcatgcccctcacggcctttgtgctgggcaaggtcttccggctgaagaacattgaggcactggccatcttggtctgtggctgctcacctggagggaacctgtccaatgtcttcagtctggccatgaagggggacatgaacctcagcattgtgatgaccacctgctccaccttctgtgcccttggcatgatgcctctcctcctgtacatctactccagggggatctatgatggggacctgaaggacaaggtgccctataaaggcatcgtgatatcactggtcctggttctcattccttgcaccatagggatcgtcctcaaatccaaacggccacaatacatgcgctatgtcatcaagggagggatgatcatcattctcttgtgcagtgtggccgtcacagttctctctgccatcaatgtggggaagagcatcatgtttgccatgacaccactcttgattgccacctcctccctgatgccttttattggctttctgctgggttatgttctctctgctctcttctgcctcaatggacggtgcagacgcactgtcagcatggagactggatgccaaaatgtccaactctgttccaccatcctcaatgtggcctttccacctgaagtcattggaccacttttcttctttcccctcctctacatgattttccagcttggagaagggcttctcctcattgccatattttggtgctatgagaaattcaagactcccaaggataaaacaaaaatgatctacacagctgccacaactgaagaaacaattccaggagctctgggaaatggcacctacaaaggggaggactgctccccttgcacagcctagcccttcccctggtggcctggattctggtcccaaagcaattctgaaagccagtgtggtaaactagagagagcagcaaaaacaccagtcttgcctgagtctttctccagcatttccagtacatctatcagaatcatcaagtcttggccgggaacacagacagggtgtctacccaagaagcctcacctatccccaacttagaatttgctacttattttaaagacttgttcagtgactgtaaactctatgaaaccagaaaccgaatctgcctcttgctgggatctctaaaagtgtctgataagcatcttaaagtcactcaattcctgaactaatcaatatatatgtttaacccattactcaaatacccaaatcccattccaagttttgtgacccaaaagagaaataaatgctcacaagtgctgtagaattaaacttcagaagttctaacctaaaaagttcagatcctattccttcccttttgacattattgggatgatgctcccgaaaagtcaaatttgacatcaagtatgcaaaagtgaacacagtaagatgcaatcaggcaaaacaaactcaaaaaatagctaatgaaatgaaaaaactgggcgaatgcatcatgttagtagaggaggaaaacttttgacaaggaaaaaccaggaaacaaacacatacattaacacaatgttacctcactaataatctcttttttaagttcagtaggtatttggttttaacacaaggcgcccccaaaactgggtacagcaaactactgccaaaatgagtcgtttcccaattcaaagaaaaatgttcaaatacctagaattcacaaatttcaaattgtctctaataaaatttaaacattttgcatatca

SEQ ID NO: 80 - DNA, 1050 bp, Homo sapiens
  source 1..1050: mol_type = genomic DNA
atggaggcccacaacgcgtctgccccattcaacttcaccctgccacccaactttggcaagcgccccacagacctggcactgagcgtcatcctggtgttcatgttgttcttcatcatgctctcgctgggctgcaccatggagttcagcaagatcaaggctcacttatggaagcctaaagggctggccatcgccctggtggcacagtatggcatcatgcccctcacggcctttgtgctgggcaaggtcttccggctgaagaacattgaggcactggccatcttggtctgtggctgctcacctggagggaacctgtccaatgtcttcagtctggccatgaagggggacatgaacctcagcattgtgatgaccacctgctccaccttctgtgcccttggcatgatgcctctcctcctgtacatctactccagggggatctatgatggggacctgaaggacaaggtgccctataaaggcatcgtgatatcactggtcctggttctcattccttgcaccatagggatcgtcctcaaatccaaacggccacaatacatgcgctatgtcatcaagggagggatgatcatcattctcttgtgcagtgtggccgtcacagttctctctgccatcaatgtggggaagagcatcatgtttgccatgacaccactcttgattgccacctcctccctgatgccttttattggctttctgctgggttatgttctctctgctctcttctgcctcaatggacggtgcagacgcactgtcagcatggagactggatgccaaaatgtccaactctgttccaccatcctcaatgtggcctttccacctgaagtcattggaccacttttcttctttcccctcctctacatgattttccagcttggagaagggcttctcctcattgccatattttggtgctatgagaaattcaagactcccaaggataaaacaaaaatgatctacacagctgccacaactgaagaaacaattccaggagctctgggaaatggcacctacaaaggggaggactgctccccttgcacagcctag

SEQ ID NO: 81 - protein, 117 aa, synthetic construct
GWSSKPRQGMGTNLSVPNPLGFFPDHQLDPAFGANSNNPDWDFNPNKDHWPEANQVGAGAFGPGFTPPHGGLLGWSPQAQGILTTVPVAPPPASTNRQSGRQPTPISPPLRDSHPQA

SEQ ID NO: 82 - protein, 116 aa, synthetic construct
WSSKPRQGMGTNLSVPNPLGFFPDHQLDPAFGANSNNPDWDFNPNKDHWPEANQVGAGAFGPGFTPPHGGLLGWSPQAQGILTTVPVAPPPASTNRQSGRQPTPISPPLRDSHPQA

SEQ ID NO: 83 - protein, 67 aa, synthetic construct
GWSSKPRQGMGTNLSVPNPLGFFPDHQLDPAFGANSNNPDWDFNPNKDHWPEANQVGAGAFGPGFTP

SEQ ID NO: 84 - protein, 66 aa, synthetic construct
WSSKPRQGMGTNLSVPNPLGFFPDHQLDPAFGANSNNPDWDFNPNKDHWPEANQVGAGAFGPGFTP

SEQ ID NO: 85 - protein, 57 aa, synthetic construct
GWSSKPRQGMGTNLSVPNPLGFFPDHQLDPAFGANSNNPDWDFNPNKDHWPEANQVG

SEQ ID NO: 86 - protein, 56 aa, synthetic construct
WSSKPRQGMGTNLSVPNPLGFFPDHQLDPAFGANSNNPDWDFNPNKDHWPEANQVG

SEQ ID NO: 87 - protein, 46 aa, synthetic construct
GWSSKPRQGMGTNLSVPNPLGFFPDHQLDPAFGANSNNPDWDFNPN

SEQ ID NO: 88 - protein, 45 aa, synthetic construct
WSSKPRQGMGTNLSVPNPLGFFPDHQLDPAFGANSNNPDWDFNPN

SEQ ID NO: 89 - protein, 106 aa, synthetic construct
TNLSVPNPLGFFPDHQLDPAFGANSNNPDWDFNPNKDHWPEANQVGAGAFGPGFTPPHGGLLGWSPQAQGILTTVPVAPPPASTNRQSGRQPTPISPPLRDSHPQA

SEQ ID NO: 90 - protein, 75 aa, synthetic construct
TNLSVPNPLGFFPDHQLDPAFGANSNNPDWDFNPNKDHWPEANQVGAGAFGPGFTPPHGGLLGWSPQAQGILTTV

SEQ ID NO: 91 - protein, 59 aa, synthetic construct
TNLSVPNPLGFFPDHQLDPAFGANSNNPDWDFNPNKDHWPEANQVGAGAFGPGFTPPHG

SEQ ID NO: 92 - protein, 54 aa, synthetic construct
TNLSVPNPLGFFPDHQLDPAFGANSNNPDWDFNPNKDHWPEANQVGAGAFGPGF

SEQ ID NO: 93 - protein, 46 aa, synthetic construct
TNLSVPNPLGFFPDHQLDPAFGANSNNPDWDFNPNKDHWPEANQVG

SEQ ID NO: 94 - protein, 43 aa, synthetic construct
TNLSVPNPLGFFPDHQLDPAFGANSNNPDWDFNPNKDHWPEAN

SEQ ID NO: 95 - protein, 42 aa, synthetic construct
TNLSVPNPLGFFPDHQLDPAFGANSNNPDWDFNPNKDHWPEA

SEQ ID NO: 96 - protein, 40 aa, synthetic construct
TNLSVPNPLGFFPDHQLDPAFGANSNNPDWDFNPNKDHWP

SEQ ID NO: 97 - protein, 35 aa, synthetic construct
TNLSVPNPLGFFPDHQLDPAFGANSNNPDWDFNPN

SEQ ID NO: 98 - protein, 34 aa, synthetic construct
TNLSVPNPLGFFPDHQLDPAFGANSNNPDWDFNP

SEQ ID NO: 99 - protein, 32 aa, synthetic construct
TNLSVPNPLGFFPDHQLDPAFGANSNNPDWDF

SEQ ID NO: 100 - protein, 29 aa, synthetic construct
TNLSVPNPLGFFPDHQLDPAFGANSNNPD

SEQ ID NO: 101 - protein, 24 aa, synthetic construct
TNLSVPNPLGFFPDHQLDPAFGAN

SEQ ID NO: 102 - protein, 19 aa, synthetic construct
TNLSVPNPLGFFPDHQLDP

SEQ ID NO: 103 - protein, 35 aa, synthetic construct
TNLSVPNPLGFFPDHQLDPAFGANSNNPDWDFNPV

SEQ ID NO: 104 - protein, 35 aa, synthetic construct
TNLSVPNPLGFFPDHQLDPAFKANSENPDWDLNPN

SEQ ID NO: 105 - protein, 36 aa, synthetic construct
GQNLSTSNPLGFFPDHQLDPAFRANTANPDWDFNPN

SEQ ID NO: 106 - protein, 35 aa, synthetic construct
KNISTTNPLGFFPDHQLDPAFRANTRNPDWDHNPN

SEQ ID NO: 107 - protein, 35 aa, synthetic construct
QNLSVPNPLGFFPDHQLDPLFRANSSSPDWDFNTN

SEQ ID NO: 108 - protein, 35 aa, synthetic construct
KNLSASNPLGFLPDHQLDPAFRANTNNPDWDFNPK

SEQ ID NO: 109 - protein, 34 aa, synthetic construct
KNLSASNPLGFLPDHQLDPAFRANTNNPDWDFNP

SEQ ID NO: 110 - protein, 35 aa, synthetic construct; identical to SEQ ID NO: 107

SEQ ID NO: 111 - protein, 35 aa, synthetic construct
TDLSVPNPLGFFPDHQLDPAFGANSNNPDWDFNPN

SEQ ID NO: 112 - protein, 35 aa, synthetic construct
TNLSVPNPLGFLPDHQLDPAFGANSNNPDWDFNPN

SEQ ID NO: 113 - protein, 35 aa, synthetic construct
TNLSVPNPLGFFPDHQLDPAFKANSNNPDWDFNPN

SEQ ID NO: 114 - protein, 35 aa, synthetic construct
TNLSVPNPLGFFPDHQLDPAFGANSENPDWDFNPN

SEQ ID NO: 115 - protein, 35 aa, synthetic construct
TNLSVPNPLGFFPDHQLDPAFGANSNNPDWDFKPN

SEQ ID NO: 116 - protein, 35 aa, synthetic construct
TNLSVPNPLGFFPDHQLDPAFGANSNNPDWDLNPN

SEQ ID NO: 117 - protein, 35 aa, synthetic construct
TNLSVPNPLGFFPDHQLDPAFGANSNNPDWDFNPH

SEQ ID NO: 118 - protein, 35 aa, synthetic construct
TNLSVPNPLGFFPDHQLDPAFGANSNNPDWDFNPY

SEQ ID NO: 119 - protein, 35 aa, synthetic construct
TNLSVPNPLGFFPDHQLDPAFGANSNNPDWDFNPK

SEQ ID NO: 120 - protein, 46 aa, synthetic construct
TNLSVPNPLGFFPDHQLDPAFGANSNNPDWDFNPNKAHWPEANQVG

SEQ ID NO: 121 - protein, 46 aa, synthetic construct
TNLSVPNPLGFFPDHQLDPAFGANSNNPDWDFNPNKDQWPEANQVG

SEQ ID NO: 122 - protein, 46 aa, synthetic construct
TNLSVPNPLGFFPDHQLDPAFGANSNNPDWDFNPNKDNWPEANQVG

SEQ ID NO: 123 - protein, 46 aa, synthetic construct
TNLSVPNPLGFFPDHQLDPAFGANSNNPDWDFNPNKDHWPKANQVG

SEQ ID NO: 124 - protein, 46 aa, synthetic construct
TNLSVPNPLGFFPDHQLDPAFGANSNNPDWDFNPNKDHWPDANQVG

SEQ ID NO: 125 - protein, 46 aa, synthetic construct
TNLSVPNPLGFFPDHQLDPAFGANSNNPDWDFNPNKDHWPESNQVG

SEQ ID NO: 126 - protein, 46 aa, synthetic construct
TNLSVPNPLGFFPDHQLDPAFGANSNNPDWDFNPNKDHWPEAKQVG

SEQ ID NO: 127 - protein, 46 aa, synthetic construct
TNLSVPNPLGFFPDHQLDPAFGANSNNPDWDFNPNKDHWPEADQVG

SEQ ID NO: 128 - protein, 46 aa, synthetic construct
TNLSVPNPLGFFPDHQLDPAFGANSNNPDWDFNPNKDHWPEANKVG

SEQ ID NO: 129 - protein, 46 aa, synthetic construct
GWSSKPRKGMGTNLSVPNPLGFFPDHQLDPAFGANSNNPDWDFNPN

SEQ ID NO: 130 - protein, 46 aa, synthetic construct; identical to SEQ ID NO: 129

SEQ ID NO: 131 - protein, 45 aa, synthetic construct
LSWTVPLEWGTNLSVPNPLGFFPDHQLDPAFGANSNNPDWDFNPN

SEQ ID NO: 132 - protein, 46 aa, synthetic construct
APLSTTRRGMGTNLSVPNPLGFFPDHQLDPAFGANSNNPDWDFNPN

SEQ ID NO: 133 - protein, 45 aa, synthetic construct; identical to SEQ ID NO: 131

SEQ ID NO: 134 - protein, 46 aa, synthetic construct
APLSTARRGMGTNLSVPNPLGFFPDHQLDPAFGANSNNPDWDFNPN

SEQ ID NO: 135 - protein, 70 aa, synthetic construct
DHWPEANQVGAGAFGPGFTPPHGGLLGWSPQAQGILTTVPVAPPPASTNRQSGRQPTPISPPLRDSHPQA

SEQ ID NO: 136 - protein, 39 aa, synthetic construct
DHWPEANQVGAGAFGPGFTPPHGGLLGWSPQAQGILTTV

SEQ ID NO: 137 - protein, 23 aa, synthetic construct
DHWPEANQVGAGAFGPGFTPPHG

SEQ ID NO: 138 - protein, 20 aa, synthetic construct
DHWPEANQVGAGAFGPGFTP

SEQ ID NO: 139 - protein, 18 aa, synthetic construct
DHWPEANQVGAGAFGPGF

SEQ ID NO: 140 - skipped

SEQ ID NO: 141 - protein, 10 aa, synthetic construct
DHWPEANQVG

SEQ ID NO: 142 - skipped

SEQ ID NO: 143 - protein, 10 aa, synthetic construct
DDWPAANQVG

SEQ ID NO: 144 - protein, 10 aa, synthetic construct
DNWPDANKVG

SEQ ID NO: 145 - protein, 10 aa, synthetic construct
DTWPDANKVG

SEQ ID NO: 146 - protein, 10 aa, synthetic construct
DHWTEANKVG

SEQ ID NO: 147 - protein, 10 aa, synthetic construct
DSWPMANKVG

SEQ ID NO: 148 - protein, 10 aa, synthetic construct
DPWPEANKVG

SEQ ID NO: 149 - protein, 10 aa, synthetic construct
DNWPMANKVG

SEQ ID NO: 150 - protein, 10 aa, synthetic construct
AHWPEANQVG

SEQ ID NO: 151 - protein, 10 aa, synthetic construct
DQWPEANQVG

SEQ ID NO: 152 - protein, 10 aa, synthetic construct
DNWPEANQVG

SEQ ID NO: 153 - protein, 10 aa, synthetic construct
DHWPKANQVG

SEQ ID NO: 154 - protein, 10 aa, synthetic construct
DHWPDANQVG

SEQ ID NO: 155 - protein, 10 aa, synthetic construct
DHWPESNQVG

SEQ ID NO: 156 - protein, 10 aa, synthetic construct
DHWPEAKQVG

SEQ ID NO: 157 - protein, 10 aa, synthetic construct
DHWPEADQVG

SEQ ID NO: 158 - protein, 10 aa, synthetic construct
DHWPEANKVG

SEQ ID NO: 159 - protein, 47 aa, synthetic construct; identical to SEQ ID NO: 30
  source 1..47: note = N-terminal modification with myristic acid and C-terminal modification with amination

SEQ ID NO: 160 - protein, 47 aa, synthetic construct; identical to SEQ ID NO: 30
  source 1..47: note = N-terminal modification with palmitic acid and C-terminal modification with amination

SEQ ID NO: 161 - protein, 47 aa, synthetic construct; identical to SEQ ID NO: 30
  source 1..47: note = N-terminal modification with stearic acid and C-terminal modification with amination

SEQ ID NO: 162 - protein, 47 aa, synthetic construct; identical to SEQ ID NO: 30
  source 1..47: note = N-terminal modification with cholesterol and C-terminal modification with amination

SEQ ID NO: 163 - protein, 47 aa, synthetic construct; identical to SEQ ID NO: 30
  source 1..47: note = N-terminal modification with PEG and C-terminal modification with amination

SEQ ID NO: 164 - protein, 47 aa, synthetic construct; identical to SEQ ID NO: 60
  source 1..47: note = N-terminal modification with myristic acid and C-terminal modification with amination

SEQ ID NO: 165 - protein, 47 aa, synthetic construct; identical to SEQ ID NO: 60
  source 1..47: note = N-terminal modification with myristic acid and C-terminal modification with amination

SEQ ID NO: 166 - protein, 44 aa, synthetic construct
  source 1..44: note = N-terminal modification with myristic acid and C-terminal modification with amination
GTNLSVPNPLGFFPDHQLDPAFGANSNNPDWDFNPNKDHWPEAK

SEQ ID NO: 167 - protein, 42 aa, synthetic construct
  source 1..42: note = N-terminal modification with myristic acid and C-terminal modification with amination
GTNLSVPNPLGFFPDHQLDPAFGANSNNPDWDFNPNKDHWPK

SEQ ID NO: 168 - protein, 37 aa, synthetic construct
  source 1..37: note = N-terminal modification with myristic acid and C-terminal modification with amination
GTNLSVPNPLGFFPDHQLDPAFGANSNNPDWDFNPNK

SEQ ID NO: 169 - protein, 36 aa, synthetic construct
  source 1..36: note = N-terminal modification with myristic acid and C-terminal modification with amination
GTNLSVPNPLGFFPDHQLDPAFGANSNNPDWDFNPK

SEQ ID NO: 170 - protein, 34 aa, synthetic construct
  source 1..34: note = N-terminal modification with myristic acid and C-terminal modification with amination
GTNLSVPNPLGFFPDHQLDPAFGANSNNPDWDFK

SEQ ID NO: 171 - protein, 37 aa, synthetic construct
  source 1..37: note = N-terminal modification with myristic acid and C-terminal modification with amination
GTNLSVPNPLGFFPDHQLDPAFGANSNNPDWDFNPVK

SEQ ID NO: 172 - protein, 37 aa, synthetic construct
  source 1..37: note = N-terminal modification with myristic acid and C-terminal modification with amination
GTNLSVPNPLGFFPDHQLDPAFKANSENPDWDLNPNK

SEQ ID NO: 173 - protein, 38 aa, synthetic construct
  source 1..38: note = N-terminal modification with myristic acid and C-terminal modification with amination
GGQNLSTSNPLGFFPDHQLDPAFRANTANPDWDFNPNK

SEQ ID NO: 174 - protein, 37 aa, synthetic construct
  source 1..37: note = N-terminal modification with myristic acid and C-terminal modification with amination
GKNISTTNPLGFFPDHQLDPAFRANTRNPDWDHNPNK

SEQ ID NO: 175 - protein, 37 aa, synthetic construct
  source 1..37: note = N-terminal modification with myristic acid and C-terminal modification with amination
GQNLSVPNPLGFFPDHQLDPLFRANSSSPDWDFNTNK

SEQ ID NO: 176 - protein, 37 aa, synthetic construct
  source 1..37: note = N-terminal modification with myristic acid and C-terminal modification with amination
GKNLSASNPLGFLPDHQLDPAFRANTNNPDWDFNPKK

SEQ ID NO: 177 - protein, 37 aa, synthetic construct; identical to SEQ ID NO: 176
  source 1..37: note = N-terminal modification with myristic acid and C-terminal modification with amination

SEQ ID NO: 178 - protein, 37 aa, synthetic construct; identical to SEQ ID NO: 175
  source 1..37: note = N-terminal modification with myristic acid and C-terminal modification with amination

SEQ ID NO: 179 - protein, 37 aa, synthetic construct
  source 1..37: note = N-terminal modification with myristic acid and C-terminal modification with amination
GFFPDHQLDPAFGANSNNPDWDFNPNKDHWPEANQVG

SEQ ID NO: 180 - protein, 28 aa, synthetic construct
  source 1..28: note = N-terminal modification with myristic acid and C-terminal modification with amination
PAFGANSNNPDWDFNPNKDHWPEANQVG

SEQ ID NO: 181 - protein, 20 aa, synthetic construct
  source 1..20: note = N-terminal modification with myristic acid and C-terminal modification with amination
NPDWDFNPNKDHWPEANQVG

SEQ ID NO: 182 - protein, 15 aa, synthetic construct
  source 1..15: note = N-terminal modification with myristic acid and C-terminal modification with amination
FNPNKDHWPEANQVG